European Patent Application EP 4 190 813 A1, published June 7, 2023. Title: ANTI-CD47 ANTIBODY AND USE THEREOF. Applicant: Bio-Thera Solutions, Ltd. Application EP21850447.0. The sequence listing filed with the application follows.

SEQUENCE LISTING (65 sequences)

SEQ ID NO: 1 - protein, 139 aa, Homo sapiens
MWPLVAALLLGSACCGSAQLLFNKTKSVEFTFCNDTVVIPCFVTNMEAQNTTEVYVKWKFKGRDIYTFDGALNKSTVPTDFSSAKIEVSQLLKGDASLKMDKSDAVSHTGNYTCEVTELTREGETIIELKYRVVSWFSP

SEQ ID NO: 2 - protein, 6 aa, Artificial Sequence
HHHHHH

SEQ ID NO: 3 - protein, 330 aa, Artificial Sequence [sequence omitted]

SEQ ID NO: 4 - protein, 327 aa, Artificial Sequence
ASTKGPSVFPLAPCSRSTSESTAALGCLVKDYFPEPVTVSWNSGALTSGVHTFPAVLQSSGLYSLSSVVTVPSSSLGTKTYTCNVDHKPSNTKVDKRVESKYGPPCPPCPAPEFLGGPSVFLFPPKPKDTLMISRTPEVTCVVVDVSQEDPEVQFNWYVDGVEVHNAKTKPREEQFNSTYRVVSVLTVLHQDWLNGKEYKCKVSNKGLPSSIEKTISKAKGQPREPQVYTLPPSQEEMTKNQVSLTCLVKGFYPSDIAVEWESNGQPENNYKTTPPVLDSDGSFFLYSRLTVDKSRWQEGNVFSCSVMHEALHNHYTQKSLSLSLGK

SEQ ID NO: 5 - protein, 107 aa, Artificial Sequence [sequence omitted]

SEQ ID NO: 6 - protein, 120 aa, Artificial Sequence
QMQLVQSGAEVKKTGSSVKVSCKASGFNIKDYYLHWVRQAPGQALEWMGWIDPDQGDTEYAQKFQDRVTITRDRSMSTAYMELSSLRSEDTAMYYCNAAYGSSSYPMDYWGQGTTVTVSS

SEQ ID NO: 7 - protein, 107 aa, Artificial Sequence
NIQMTQSPSAMSASVGDRVTITCKASQDIHRYLSWFQQKPGKVPKHLIYRANRLVSGVPSRFSGSGSGTEFTLTISSLQPEDFATYYCLQYDEFPYTFGGGTKVEIK

SEQ ID NO: 8 - protein, 117 aa, Artificial Sequence
QVQLVQSGAEVKKPGASVKVSCKASGYTFTNYNMHWVRQAPGQRLEWMGTIYPGNDDTSYNQKFKDRVTITADTSASTAYMELSSLRSEDTAVYYCARGGYRAMDYWGQGTLVTVSS

SEQ ID NO: 9 - protein, 112 aa, Artificial Sequence
DIVMTQSPLSLPVTPGEPASISCRSSQSIVYSNGNTYLGWYLQKPGQSPQLLIYKVSNRFSGVPDRFSGSGSGTDFTLKISRVEAEDVGVYYCFQGSHVPYTFGQGTKLEIK

SEQ ID NO: 10 - protein, 15 aa, Artificial Sequence
GGGGSGGGGSGGGGS

SEQ ID NO: 11 - protein, 116 aa, Artificial Sequence
QVQLQESGPGLVKPSETLSLTCTVSGGSLDNYYWSWIRQPPGKGLEWIGYIYYSGNTNYNPSLKSRVTISVDTSKNQFSLRLRSVTAADTAVYYCARGGRFLERYWGQGTLVTVSS

SEQ ID NO: 12 - protein, 107 aa, Artificial Sequence
DIQMTQSPSSVSASVGDRVTISCRANQAIGTWLAWYQQKPGKAPKLLIYAASTLQSGVPSRFSGSGSGTEFTLTISSLQAEDVAVYYCQQYYTTPLTFGGGTKLEIK

SEQ ID NO: 13 - protein, 107 aa, Artificial Sequence
EIVLTQPPSSLSASVGDRVTIPCRASLSIGSFLNWYQQRPGEAPKLLIFAASSLRSGVPSRFSGSGSGTDFTLTISGLQPEDFATYYCQQTYTTPYTFGQGTKVDIK

SEQ ID NO: 14 - protein, 6 aa, Artificial Sequence
DNYYWS

SEQ ID NO: 15 - protein, 6 aa, Artificial Sequence
DGYYWS

SEQ ID NO: 16 - protein, 6 aa, Artificial Sequence
NDYYWS

SEQ ID NO: 17 - protein, 16 aa, Artificial Sequence
YIYYSGNTNYNPSLKS

SEQ ID NO: 18 - protein, 16 aa, Artificial Sequence
RIYGNSTTNYNPSLKS

SEQ ID NO: 19 - protein, 16 aa, Artificial Sequence
RIYGNGDTNYNPSLKS

SEQ ID NO: 20 - protein, 16 aa, Artificial Sequence
RIYYNGNTNYNPSLKS

SEQ ID NO: 21 - protein, 16 aa, Artificial Sequence
RIYGDSATNYNPSLKS

SEQ ID NO: 22 - protein, 16 aa, Artificial Sequence
RIYDGSGTNYNPSLKS

SEQ ID NO: 23 - protein, 8 aa, Artificial Sequence
GGRFLERY

SEQ ID NO: 24 - protein, 8 aa, Artificial Sequence
GGRIFGGY

SEQ ID NO: 25 - protein, 8 aa, Artificial Sequence
GGRIFAGY

SEQ ID NO: 26 - protein, 8 aa, Artificial Sequence
GGRILAGY

SEQ ID NO: 27 - protein, 8 aa, Artificial Sequence
GGRIFSGY

SEQ ID NO: 28 - protein, 7 aa, Artificial Sequence
GRGIFGY

SEQ ID NO: 29 - protein, 7 aa, Artificial Sequence
GGRIFGH

SEQ ID NO: 30 - protein, 11 aa, Artificial Sequence
RASLSIGSFLN

SEQ ID NO: 31 - protein, 11 aa, Artificial Sequence
RANQAIGTWLA

SEQ ID NO: 32 - protein, 7 aa, Artificial Sequence
AASSLRS

SEQ ID NO: 33 - protein, 7 aa, Artificial Sequence
AASTLQS

SEQ ID NO: 34 - protein, 9 aa, Artificial Sequence
QQTYTTPYT

SEQ ID NO: 35 - protein, 9 aa, Artificial Sequence
QQYYTTPLT

SEQ ID NO: 36 - protein, 116 aa, Artificial Sequence
QVQLQESGPGLVKPSETLSLTCTVSGGSLDNYYWSWIRQPPGKGLEWIGYIYYSGNTNYNPSLKSRVTISVDTSKNQFSLRLRSVTAADTAVYYCARGGRIFGGYWGQGTLVTVSS

SEQ ID NO: 37 - protein, 116 aa, Artificial Sequence
QVQLQESGPGLVKPSETLSLTCTVSGGSLDNYYWSWIRQPPGKGLEWIGYIYYSGNTNYNPSLKSRVTISVDTSKNQFSLRLRSVTAADTAVYYCARGGRIFAGYWGQGTLVTVSS

SEQ ID NO: 38 - protein, 116 aa, Artificial Sequence
QVQLQESGPGLVKPSETLSLTCTVSGGSLDGYYWSWIRQPPGKGLEWIGRIYGNSTTNYNPSLKSRVTISVDTSKNQFSLRLRSVTAADTAVYYCARGGRIFAGYWGQGTLVTVSS

SEQ ID NO: 39 - protein, 116 aa, Artificial Sequence
QVQLQESGPGLVKPSETLSLTCTVSGGSLNDYYWSWIRQPPGKGLEWIGRIYGNGDTNYNPSLKSRVTISVDTSKNQFSLRLRSVTAADTAVYYCARGGRILAGYWGQGTLVTVSS

SEQ ID NO: 40 - protein, 116 aa, Artificial Sequence
QVQLQESGPGLVKPSETLSLTCTVSGGSLDNYYWSWIRQPPGKGLEWIGRIYYNGNTNYNPSLKSRVTISVDTSKNQFSLRLRSVTAADTAVYYCARGGRILAGYWGQGTLVTVSS

SEQ ID NO: 41 - protein, 116 aa, Artificial Sequence
QVQLQESGPGLVKPSETLSLTCTVSGGSLDNYYWSWIRQPPGKGLEWIGYIYYSGNTNYNPSLKSRVTISVDTSKNQFSLRLRSVTAADTAVYYCARGGRIFSGYWGQGTLVTVSS

SEQ ID NO: 42 - protein, 115 aa, Artificial Sequence
QVQLQESGPGLVKPSETLSLTCTVSGGSLDNYYWSWIRQPPGKGLEWIGYIYYSGNTNYNPSLKSRVTISVDTSKNQFSLRLRSVTAADTAVYYCARGRGIFGYWGQGTLVTVSS

SEQ ID NO: 43 - protein, 116 aa, Artificial Sequence
QVQLQESGPGLVKPSETLSLTCTVSGGSLDNYYWSWIRQPPGKGLEWIGRIYGDSATNYNPSLKSRVTISVDTSKNQFSLRLRSVTAADTAVYYCARGGRIFSGYWGQGTLVTVSS

SEQ ID NO: 44 - protein, 115 aa, Artificial Sequence
QVQLQESGPGLVKPSETLSLTCTVSGGSLDNYYWSWIRQPPGKGLEWIGYIYYSGNTNYNPSLKSRVTISVDTSKNQFSLRLRSVTAADTAVYYCARGGRIFGHWGQGTLVTVSS

SEQ ID NO: 45 - protein, 107 aa, Artificial Sequence
EIVLTQSPSTLSASVGDRVTIPCRASLSIGSFLNWYQQRPGEAPKLLIFAASSLRSGVPSRFSGSGSGTDFTLTISGLQPEDFATYYCQQTYTTPYTFGQGTKVEIK

SEQ ID NO: 46 - protein, 107 aa, Artificial Sequence
DIVMTQSPSSLSASVGDRVTIPCRASLSIGSFLNWYQQRPGEAPKLLIFAASSLRSGVPSRFSGSGSGTDFTLTISGLQPEDFATYYCQQTYTTPYTFGPGTRLDIK

SEQ ID NO: 47 - protein, 107 aa, Artificial Sequence
EIVLTQSPSSLSASVGDRVTIPCRASLSIGSFLNWYQQRPGEAPKLLIFAASSLRSGVPSRFSGSGSGTDFTLTISGLQPEDFATYYCQQTYTTPYTFGPGTRLEIK

SEQ ID NO: 48 - protein, 107 aa, Artificial Sequence
DIQMTQSPSSLSASVGDRVTIPCRASLSIGSFLNWYQQRPGEAPKLLIFAASSLRSGVPSRFSGSGSGTDFTLTISSLQPEDFATYYCQQTYTTPYTFGQGTKVEIK

SEQ ID NO: 49 - protein, 107 aa, Artificial Sequence
EIVLTQSPSSLSASVGDRVTIPCRASLSIGSFLNWYQQRPGEAPKLLIFAASSLRSGVPSRFSGSGSGTDFTLTISSLQPEDFATYYCQQTYTTPYTFGQGTKLEIK

SEQ ID NO: 50 - protein, 116 aa, Artificial Sequence
QVQLQESGPGLVKPSETLSLTCTVSGGSLDNYYWSWIRQPPGKGLEWIGYIYYSGNTNYNPSLKSRVTISVDTSKNQFSLKLSSVTAADTAVYYCARGGRFLERYWGQGTLVTVSS

SEQ ID NO: 51 - protein, 107 aa, Artificial Sequence
EIVLTQSPSSLSASVGDRVTIPCRASLSIGSFLNWYQQRPGEAPKLLIFAASSLRSGVPSRFSGSGSGTDFTLTISSLQPEDFATYYCQQTYTTPYTFGQGTKVEIK

SEQ ID NO: 52 - protein, 107 aa, Artificial Sequence
EIVLTQSPSSLSASVGDRVTIPCRASLSIGSFLNWYQQKPGKAPKLLIFAASSLRSGVPSRFSGSGSGTDFTLTISSLQPEDFATYYCQQTYTTPYTFGQGTKVEIK

SEQ ID NO: 53 - protein, 107 aa, Artificial Sequence
EIVLTQSPSSLSASVGDRVTITCRASLSIGSFLNWYQQKPGKAPKLLIFAASSLRSGVPSRFSGSGSGTDFTLTISSLQPEDFATYYCQQTYTTPYTFGQGTKVEIK

SEQ ID NO: 54 - protein, 107 aa, Artificial Sequence
EIVLTQSPSSLSASVGDRVTITCRASLSIGSFLNWYQQKPGKAPKLLIYAASSLRSGVPSRFSGSGSGTDFTLTISSLQPEDFATYYCQQTYTTPYTFGQGTKVEIK

SEQ ID NO: 55 - protein, 107 aa, Artificial Sequence
DIQMTQSPSSLSASVGDRVTITCRASLSIGSFLNWYQQKPGKAPKLLIYAASSLRSGVPSRFSGSGSGTDFTLTISSLQPEDFATYYCQQTYTTPYTFGQGTKVEIK

SEQ ID NO: 56 - protein, 116 aa, Artificial Sequence
QVQLQESGPGLVKPSETLSLTCTVSGGSLDGYYWSWIRQPPGKGLEWIGRIYDGSGTNYNPSLKSRVTISVDTSKNQFSLRLRSVTAADTAVYYCARGGRIFGGYWGQGTLVTVSS

SEQ ID NO: 57 - DNA, 1329 bp, Artificial Sequence
caggtgcagctgcaggagtccggccctggcctggtgaagccttccgagaccctgtccctgacctgtaccgtgagcggcggcagcctggataactattactggagctggatccggcagcctcctggcaagggcctggagtggatcggctacatctactattccggcaacaccaattacaacccttccctgaagagccgggtgaccatctccgtggacaccagcaagaaccagtttagcctgaagctgtcctccgtgaccgccgctgataccgccgtgtactactgtgccaggggcggccggttcctggagagatattggggccagggtaccctcgtgaccgtgtccagcgctagcaccaagggcccttccgtgttccccctggccccctgtagccggtccacctctgagagcaccgctgctctgggctgtctggtgaaggattactttcccgaaccggtgaccgtgtcatggaactccggggctctgacatccggtgtccacacttttcctgcagtgctgcagtcatccggcctgtacagcctgagctctgtggtcacagtcccaagttcatccctgggaaccaagacatatacttgcaacgtggatcataaacccagcaatactaaggtcgacaaacgagtggagtctaagtacggaccaccttgcccaccatgtccagcacctgagttcctgggaggaccaagcgtgttcctgtttcctccaaagcctaaagataccctgatgatcagtcggactcccgaggtcacctgcgtggtcgtggacgtgtcccaggaggaccctgaagtccagttcaactggtacgtggacggcgtcgaagtgcacaatgctaagacaaaacctcgagaggaacagtttaactccacataccgtgtcgtgagcgtcctgactgtgctgcatcaggattggctgaacggcaaggagtataagtgcaaagtgagcaataagggactgccaagctctatcgagaaaactatttctaaggctaaaggacagcctagggaaccacaggtgtacaccctgccccctagtcaggaggaaatgactaagaaccaggtctcactgacctgtctggtgaaagggttctatccttcagatattgcagtggagtgggaatccaatggtcagccagagaacaattacaagacaactccacccgtgctggacagcgatgggtctttctttctgtattctagactgaccgtggacaaaagtcgctggcaggagggtaatgtcttttcttgtagtgtgatgcacgaagccctgcacaaccactacactcagaaaagcctgtcactgtccctgggtaaa

SEQ ID NO: 58 - DNA, 645 bp, Artificial Sequence
gagatcgtgctgacccagtccccctccagcctgagcgccagcgtgggagaccgggtgaccatcccctgccgggcttccctgtccatcggcagcttcctgaactggtatcagcagaggcctggcgaggcccctaagctgctgatctttgccgcttccagcctgcggagcggcgtgcctagcaggttctccggcagcggctccggcaccgatttcaccctgaccatcagcggcctgcagcccgaggatttcgccacctactactgccagcagacctacaccaccccttacacctttggccagggcaccaaggtggacatcaagcgtacggtggctgcaccatctgtcttcatcttcccgccatctgatgagcagttgaaatctggaactgcctctgttgtgtgcctgctgaataacttctatcccagagaggccaaagtacagtggaaggtggataacgccctccaatcgggtaactcccaggagagtgtcacagagcaggacagcaaggacagcacctacagcctcagcagcaccctgacgctgagcaaagcagactacgagaaacacaaagtctacgcctgcgaagtcacccatcagggcctgagctcgcccgtcacaaagagcttcaacaggggagagtgttga

SEQ ID NO: 59 - DNA, 714 bp, Artificial Sequence
caggtgcagctgcaggagtcgggcccaggactggtgaagccttcggagaccctgtccctcacctgcactgtctctggtggctccctcgataattactactggagctggatccggcagcccccagggaagggactggagtggattggatatatctattacagtgggaacaccaactacaacccctccctcaagagtcgagtcaccatatcagtagacacgtccaagaaccagttctcgttgaggctgaggtctgtgaccgctgcggacacggccgtgtattactgtgcgagaggagggcgatttttggaacgttactggggccagggaaccctggtcaccgtctcctcaggtggaggcggttcaggcggaggtggctctggcggtggcggatcggacatccagatgacccagtctccatcttccgtgtctgcatctgtaggagacagagtcaccatctcttgtcgggcgaatcaggctattggcacttggttagcctggtatcagcaaaagccaggaaaagcccctaagctcctgatctatgcggcatccactttgcaaagtggggtcccatcaaggttcagcggcagtggatctgggacagaattcactctcaccatcagcagcctgcaggctgaagatgtggcagtttattactgtcagcaatattatactactcccctcactttcggcggagggaccaagctggagatcaaa

SEQ ID NO: 60 - protein, 443 aa, Artificial Sequence
QVQLQESGPGLVKPSETLSLTCTVSGGSLDNYYWSWIRQPPGKGLEWIGYIYYSGNTNYNPSLKSRVTISVDTSKNQFSLKLSSVTAADTAVYYCARGGRFLERYWGQGTLVTVSSASTKGPSVFPLAPCSRSTSESTAALGCLVKDYFPEPVTVSWNSGALTSGVHTFPAVLQSSGLYSLSSVVTVPSSSLGTKTYTCNVDHKPSNTKVDKRVESKYGPPCPPCPAPEFLGGPSVFLFPPKPKDTLMISRTPEVTCVVVDVSQEDPEVQFNWYVDGVEVHNAKTKPREEQFNSTYRVVSVLTVLHQDWLNGKEYKCKVSNKGLPSSIEKTISKAKGQPREPQVYTLPPSQEEMTKNQVSLTCLVKGFYPSDIAVEWESNGQPENNYKTTPPVLDSDGSFFLYSRLTVDKSRWQEGNVFSCSVMHEALHNHYTQKSLSLSLGK

SEQ ID NO: 61 - protein, 214 aa, Artificial Sequence
EIVLTQSPSSLSASVGDRVTIPCRASLSIGSFLNWYQQRPGEAPKLLIFAASSLRSGVPSRFSGSGSGTDFTLTISGLQPEDFATYYCQQTYTTPYTFGQGTKVDIKRTVAAPSVFIFPPSDEQLKSGTASVVCLLNNFYPREAKVQWKVDNALQSGNSQESVTEQDSKDSTYSLSSTLTLSKADYEKHKVYACEVTHQGLSSPVTKSFNRGEC

SEQ ID NO: 62 - protein, 446 aa, Artificial Sequence
QVQLQESGPGLVKPSETLSLTCTVSGGSLDNYYWSWIRQPPGKGLEWIGYIYYSGNTNYNPSLKSRVTISVDTSKNQFSLKLSSVTAADTAVYYCARGGRFLERYWGQGTLVTVSSASTKGPSVFPLAPSSKSTSGGTAALGCLVKDYFPEPVTVSWNSGALTSGVHTFPAVLQSSGLYSLSSVVTVPSSSLGTQTYICNVNHKPSNTKVDKKVEPKSCDKTHTCPPCPAPELLGGPSVFLFPPKPKDTLMISRTPEVTCVVVDVSHEDPEVKFNWYVDGVEVHNAKTKPREEQYNSTYRVVSVLTVLHQDWLNGKEYKCKVSNKALPAPIEKTISKAKGQPREPQVYTLPPSRDELTKNQVSLTCLVKGFYPSDIAVEWESNGQPENNYKTTPPVLDSDGSFFLYSKLTVDKSRWQQGNVFSCSVMHEALHNHYTQKSLSLSPGK

SEQ ID NO: 63 - protein, 446 aa, Artificial Sequence
QVQLQESGPGLVKPSETLSLTCTVSGGSLDNYYWSWIRQPPGKGLEWIGYIYYSGNTNYNPSLKSRVTISVDTSKNQFSLRLRSVTAADTAVYYCARGGRFLERYWGQGTLVTVSSASTKGPSVFPLAPSSKSTSGGTAALGCLVKDYFPEPVTVSWNSGALTSGVHTFPAVLQSSGLYSLSSVVTVPSSSLGTQTYICNVNHKPSNTKVDKKVEPKSCDKTHTCPPCPAPELLGGPSVFLFPPKPKDTLMISRTPEVTCVVVDVSHEDPEVKFNWYVDGVEVHNAKTKPREEQYNSTYRVVSVLTVLHQDWLNGKEYKCKVSNKALPAPIEKTISKAKGQPREPQVYTLPPSRDELTKNQVSLTCLVKGFYPSDIAVEWESNGQPENNYKTTPPVLDSDGSFFLYSKLTVDKSRWQQGNVFSCSVMHEALHNHYTQKSLSLSPGK

SEQ ID NO: 64 - protein, 214 aa, Artificial Sequence
DIQMTQSPSSVSASVGDRVTISCRANQAIGTWLAWYQQKPGKAPKLLIYAASTLQSGVPSRFSGSGSGTEFTLTISSLQAEDVAVYYCQQYYTTPLTFGGGTKLEIKRTVAAPSVFIFPPSDEQLKSGTASVVCLLNNFYPREAKVQWKVDNALQSGNSQESVTEQDSKDSTYSLSSTLTLSKADYEKHKVYACEVTHQGLSSPVTKSFNRGEC

SEQ ID NO: 65 - protein, 107 aa, Artificial Sequence
EIVLTQSPSSLSASVGDRVTIPCRASLSIGSFLNWYQQRPGEAPKLLIFAASSLRSGVPSRFSGSGSGTDFTLTISGLQPEDFATYYCQQTYTTPYTFGQGTKVDIK